European Patent Application EP 4 644 413 A1, published November 5, 2025. Title: BINDING AGENTS HAVING ALTERED FC-MEDIATED EFFECTOR FUNCTIONS. Applicant: GENMAB BV. The sequence listing filed with the application follows.

SEQUENCE LISTING (36 sequences)

SEQ ID NO: 1 - protein, 329 aa, Homo sapiens
ASTKGPSVFPLAPSSKSTSGGTAALGCLVKDYFPEPVTVSWNSGALTSGVHTFPAVLQSSGLYSLSSVVTVPSSSLGTQTYICNVNHKPSNTKVDKRVEPKSCDKTHTCPPCPAPELLGGPSVFLFPPKPKDTLMISRTPEVTCVVVDVSHEDPEVKFNWYVDGVEVHNAKTKPREEQYNSTYRVVSVLTVLHQDWLNGKEYKCKVSNKALPAPIEKTISKAKGQPREPQVYTLPPSREEMTKNQVSLTCLVKGFYPSDIAVEWESNGQPENNYKTTPPVLDSDGSFFLYSKLTVDKSRWQQGNVFSCSVMHEALHNHYTQKSLSLSPG

SEQ ID NO: 2 - protein, 107 aa, Homo sapiens [sequence omitted]

SEQ ID NO: 3 - protein, 106 aa, Homo sapiens
GQPKAAPSVTLFPPSSEELQANKATLVCLISDFYPGAVTVAWKADSSPVKAGVETTTPSKQSNNKYAASSYLSLTPEQWKSHRSYSCQVTHEGSTVEKTVAPTECS

SEQ ID NO: 4 - protein, 329 aa, synthetic construct
ASTKGPSVFPLAPSSKSTSGGTAALGCLVKDYFPEPVTVSWNSGALTSGVHTFPAVLQSSGLYSLSSVVTVPSSSLGTQTYICNVNHKPSNTKVDKRVEPKSCDKTHTCPPCPAPELLGGPSVFLFPPKPKDTLMISRTPEVTCVVVDVSHEDPEVKFNWYVDGVEVHNAKTKPREEQYNSTYRVVSVLTVLHQDWLNGKEYKCKVSNKALPAPIEKTISKAKGQPREPQVYTLPPSRKEMTKNQVSLTCLVKGFYPSDIAVEWESNGQPENNYDTTPPVLKSDGSFFLYSDLTVDKSRWQQGNVFSCSVMHEALHNHYTQKSLSLSPG

SEQ ID NO: 5 - protein, 329 aa, synthetic construct
ASTKGPSVFPLAPSSKSTSGGTAALGCLVKDYFPEPVTVSWNSGALTSGVHTFPAVLQSSGLYSLSSVVTVPSSSLGTQTYICNVNHKPSNTKVDKRVEPKSCDKTHTCPPCPAPELLGGPSVFLFPPKPKDTLMISRTPEVTCVVVDVSHEDPEVKFNWYVDGVEVHNAKTKPREEQYNSTYRVVSVLTVLHQDWLNGKEYKCKVSNKALPAPIEKTISKAKGQPREPQVYTLPPSRKEMTKNQVSLTCLVKGFYPSDIAVEWESNGQPENNYETTPPVLKSDGSFFLYSDLTVDKSRWQQGNVFSCSVMHEALHNHYTQKSLSLSPG

SEQ ID NO: 6 - protein, 329 aa, synthetic construct
ASTKGPSVFPLAPSSKSTSGGTAALGCLVKDYFPEPVTVSWNSGALTSGVHTFPAVLQSSGLYSLSSVVTVPSSSLGTQTYICNVNHKPSNTKVDKRVEPKSCDKTHTCPPCPAPELLGGPSVFLFPPKPKDTLMISRTPEVTCVVVDVSHEDPEVKFNWYVDGVEVHNAKTKPREEQYNSTYRVVSVLTVLHQDWLNGKEYKCKVSNKALPAPIEKTISKAKGQPREPQVYTLPPSREQMTKNQVKLTCDVSGFYPSDIAVEWESNGQPENNYKTTPPVLDSDGSFFLYSKLTVDKSRWQQGNVFSCSVMHEALHNHYTQKSLSLSPG

SEQ ID NO: 7 - protein, 329 aa, synthetic construct
ASTKGPSVFPLAPSSKSTSGGTAALGCLVKDYFPEPVTVSWNSGALTSGVHTFPAVLQSSGLYSLSSVVTVPSSSLGTQTYICNVNHKPSNTKVDKRVEPKSCDKTHTCPPCPAPELLGGPSVFLFPPKPKDTLMISRTPEVTCVVVDVSHEDPEVKFNWYVDGVEVHNAKTKPREEQYNSTYRVVSVLTVLHQDWLNGKEYKCKVSNKALPAPIEKTISKAKGQPREPQVYVYPPSREEMTKNQVSLLCLVKGFYPSDIAVEWESNGQPENNYLTWPPVLDSDGSFALVSKLTVDKSRWQQGNVFSCSVMHEALHNHYTQKSLSLSPG

SEQ ID NO: 8 - protein, 329 aa, synthetic construct
ASTKGPSVFPLAPSSKSTSGGTAALGCLVKDYFPEPVTVSWNSGALTSGVHTFPAVLQSSGLYSLSSVVTVPSSSLGTQTYICNVNHKPSNTKVDKRVEPKSCDKTHTCPPCPAPELLGGPSVFLFPPKPKDTLMISRTPEVTCVVVDVSHEDPEVKFNWYVDGVEVHNAKTKPREEQYNSTYRVVSVLTVLHQDWLNGKEYKCKVSNKALPAPIEKTISKAKGQPREPRVYTLPPSREEMTENQVSLTCLVKGFYPSDIAVEWESNGQPENNYKTTPPVLVSDGSFTLYSWLTVDKSRWQQGNVFSCSVMHEALHNHYTQKSLSLSPG

SEQ ID NO: 9 - protein, 329 aa, synthetic construct
ASTKGPSVFPLAPSSKSTSGGTAALGCLVKDYFPEPVTVSWNSGALTSGVHTFPAVLQSSGLYSLSSVVTVPSSSLGTQTYICNVNHKPSNTKVDKRVEPKSCDKTHTCPPCPAPELLGGPSVFLFPPKPKDTLMISRTPEVTCVVVDVSHEDPEVKFNWYVDGVEVHNAKTKPREEQYNSTYRVVSVLTVLHQDWLNGKEYKCKVSNKALPAPIEKTISKAKGQPRRPRVYTLPPSREEMTDNQVSLVCLVKGFYPSDIAVEWESNGQPENNYKTTPPVLMSDGSFFLASVLTVDKSRWQQGNVFSCSVMHEALHNHYTQKSLSLSPG

SEQ ID NO: 10 - protein, 329 aa, synthetic construct
ASTKGPSVFPLAPSSKSTSGGTAALGCLVKDYFPEPVTVSWNSGALTSGVHTFPAVLQSSGLYSLSSVVTVPSSSLGTQTYICNVNHKPSNTKVDKRVEPKSCDKTHTCPPCPAPELLGGPSVFLFPPKPKDTLMISRTPEVTCVVVDVSHEDPEVKFNWYVDGVEVHNAKTKPREEQYNSTYRVVSVLTVLHQDWLNGKEYKCKVSNKALPAPIEKTISKAKGQPREPRVYTLPPSREEMTDNQVSLVCLVKGFYPSDIAVEWESNGQPENNYKTTPPVLMSDGSFFLASVLTVDKSRWQQGNVFSCSVMHEALHNHYTQKSLSLSPG

SEQ ID NO: 11 - protein, 329 aa, synthetic construct
ASTKGPSVFPLAPSSKSTSGGTAALGCLVKDYFPEPVTVSWNSGALTSGVHTFPAVLQSSGLYSLSSVVTVPSSSLGTQTYICNVNHKPSNTKVDKRVEPKSCDKTHTCPPCPAPELLGGPSVFLFPPKPKDTLMISRTPEVTCVVVDVSHEDPEVKFNWYVDGVEVHNAKTKPREEQYNSTYRVVSVLTVLHQDWLNGKEYKCKVSNKALPAPIEKTISKAKGQPREPQVYTKPPSREEMTKNQVSLTCLVKGFYPSDIAVEWESNGQPENNYKTTPPVLKSDGSFFLYSDLTVDKSRWQQGNVFSCSVMHEALHNHYTQKSLSLSPG

SEQ ID NO: 12 - protein, 329 aa, synthetic construct
ASTKGPSVFPLAPSSKSTSGGTAALGCLVKDYFPEPVTVSWNSGALTSGVHTFPAVLQSSGLYSLSSVVTVPSSSLGTQTYICNVNHKPSNTKVDKRVEPKSCDKTHTCPPCPAPELLGGPSVFLFPPKPKDTLMISRTPEVTCVVVDVSHEDPEVKFNWYVDGVEVHNAKTKPREEQYNSTYRVVSVLTVLHQDWLNGKEYKCKVSNKALPAPIEKTISKAKGQPREPQVYTDPPSRKEMTKNQVSLKCLVKGFYPSDIAVEWESNGQPENNYKTTPPVLDSDGSFFLYSKLTVDKSRWQQGNVFSCSVMHEALHNHYTQESLSLSPG

SEQ ID NO: 13 - protein, 329 aa, synthetic construct
ASTKGPSVFPLAPSSKSTSGGTAALGCLVKDYFPEPVTVSWNSGALTSGVHTFPAVLQSSGLYSLSSVVTVPSSSLGTQTYICNVNHKPSNTKVDKRVEPKSCDKTHTCPPCPAPELLGGPSVFLFPPKPKDTLMISRTPEVTCVVVDVSHEDPEVKFNWYVDGVEVHNAKTKPREEQYNSTYRVVSVLTVLHQDWLNGKEYKCKVSNKALPAPIEKTISKAKGQPREPKVYTDPPSREEMTENQVSLKCLVKGFYPSDIAVEWESNGQPENNYKTTPPVLDSDGSFFLYSKLTVDKSRWQQGNVFSCSVMHEALHNHYTQKSLSLSPG

SEQ ID NO: 14 - protein, 329 aa, synthetic construct
ASTKGPSVFPLAPSSKSTSGGTAALGCLVKDYFPEPVTVSWNSGALTSGVHTFPAVLQSSGLYSLSSVVTVPSSSLGTQTYICNVNHKPSNTKVDKRVEPKSCDKTHTCPPCPAPELLGGPSVFLFPPKPKDTLMISRTPEVTCVVVDVSHEDPEVKFNWYVDGVEVHNAKTKPREEQYNSTYRVVSVLTVLHQDWLNGKEYKCKVSNKALPAPIEKTISKAKGQPREPQVYTLPPSREEMTKNQVWLTCLVAGFYPSDIAVEWESNGQPENNYDTTPPVLKSDGSFFLYSKLTVDKSRWQQGNVFSCSVMHEALHNHYTQKSLSLSPG

SEQ ID NO: 15 - protein, 329 aa, synthetic construct
ASTKGPSVFPLAPSSKSTSGGTAALGCLVKDYFPEPVTVSWNSGALTSGVHTFPAVLQSSGLYSLSSVVTVPSSSLGTQTYICNVNHKPSNTKVDKRVEPKSCDKTHTCPPCPAPELLGGPSVFLFPPKPKDTLMISRTPEVTCVVVDVSHEDPEVKFNWYVDGVEVHNAKTKPREEQYNSTYRVVSVLTVLHQDWLNGKEYKCKVSNKALPAPIEKTISKAKGQPREPQVYTLPPSRKEMTKNQVSLTCLVKGFYPSDIAVEWESNGQPENNYKTTPPVLVSDGSFFLYSWLTVDKSRWQQGNVFSCSVMHEALHNHYTQESLSLSPG

SEQ ID NO: 16 - protein, 329 aa, synthetic construct
ASTKGPSVFPLAPSSKSTSGGTAALGCLVKDYFPEPVTVSWNSGALTSGVHTFPAVLQSSGLYSLSSVVTVPSSSLGTQTYICNVNHKPSNTKVDKRVEPKSCDKTHTCPPCPAPELLGGPSVFLFPPKPKDTLMISRTPEVTCVVVDVSHEDPEVKFNWYVDGVEVHNAKTKPREEQYNSTYRVVSVLTVLHQDWLNGKEYKCKVSNKALPAPIEKTISKAKGQPREPQVYTDPPSREEMTKNQVSLKCLVKGFYPSDIAVEWESNGQPENNYDTTPPVLKSDGSFFLYSDLTVDKSRWQQGNVFSCSVMHEALHNHYTQKSLSLSPG

SEQ ID NO: 17 - protein, 329 aa, synthetic construct
ASTKGPSVFPLAPSSKSTSGGTAALGCLVKDYFPEPVTVSWNSGALTSGVHTFPAVLQSSGLYSLSSVVTVPSSSLGTQTYICNVNHKPSNTKVDKRVEPKSCDKTHTCPPCPAPELLGGPSVFLFPPKPKDTLMISRTPEVTCVVVDVSHEDPEVKFNWYVDGVEVHNAKTKPREEQYNSTYRVVSVLTVLHQDWLNGKEYKCKVSNKALPAPIEKTISKAKGQPREPKVYTDPPSREKMTENQVSLKCLVEGFYPSDIAVEWESNGQPENNYKTTPPVLDSDGSFFLYSKLTVDKSRWQQGNVFSCSVMHEALHNHYTQKSLSLSPG

SEQ ID NO: 18 - protein, 329 aa, synthetic construct
ASTKGPSVFPLAPSSKSTSGGTAALGCLVKDYFPEPVTVSWNSGALTSGVHTFPAVLQSSGLYSLSSVVTVPSSSLGTQTYICNVNHKPSNTKVDKRVEPKSCDKTHTCPPCPAPELLGGPSVFLFPPKPKDTLMISRTPEVTCVVVDVSHEDPEVKFNWYVDGVEVHNAKTKPREEQYNSTYRVVSVLTVLHQDWLNGKEYKCKVSNKALPAPIEKTISKAKGQPREPQVYTLPPSRKEMTKNQVSLTCLVKGFYPSDIAVEWESNGQPENNYDTTPPVLVSDGSFFLYSWLTVDKSRWQQGNVFSCSVMHEALHNHYTQESLSLSPG

SEQ ID NO: 19 - protein, 329 aa, synthetic construct
ASTKGPSVFPLAPSSKSTSGGTAALGCLVKDYFPEPVTVSWNSGALTSGVHTFPAVLQSSGLYSLSSVVTVPSSSLGTQTYICNVNHKPSNTKVDKRVEPKSCDKTHTCPPCPAPELLGGPSVFLFPPKPKDTLMISRTPEVTCVVVDVSHEDPEVKFNWYVDGVEVHNAKTKPREEQYNSTYRVVSVLTVLHQDWLNGKEYKCKVSNKALPAPIEKTISKAKGQPREPKVYTEPPSREKMTENQVKLTCDVEGFYPSDIAVEWESNGQPENNYKTTPPVLDSDGSFFLYSKLTVDKSRWQQGNVFSCSVMHEALHNHYTQKSLSLSPG

SEQ ID NO: 20 - protein, 329 aa, synthetic construct
ASTKGPSVFPLAPSSKSTSGGTAALGCLVKDYFPEPVTVSWNSGALTSGVHTFPAVLQSSGLYSLSSVVTVPSSSLGTQTYICNVNHKPSNTKVDKRVEPKSCDKTHTCPPCPAPELLGGPSVFLFPPKPKDTLMISRTPEVTCVVVDVSHEDPEVKFNWYVDGVEVHNAKTKPREEQYNSTYRVVSVLTVLHQDWLNGKEYKCKVSNKALPAPIEKTISKAKGQPREPKVYTLPPSREEMTENQVSLTCLVKGFYPSDIAVEWESNGQPENNYKTTPPVLVSDGSFFLYSWLTVDKSRWQQGNVFSCSVMHEALHNHYTQKSLSLSPG

SEQ ID NO: 21 - protein, 329 aa, synthetic construct
ASTKGPSVFPLAPSSKSTSGGTAALGCLVKDYFPEPVTVSWNSGALTSGVHTFPAVLQSSGLYSLSSVVTVPSSSLGTQTYICNVNHKPSNTKVDKRVEPKSCDKTHTCPPCPAPELLGGPSVFLFPPKPKDTLMISRTPEVTCVVVDVSHEDPEVKFNWYVDGVEVHNAKTKPREEQYNSTYRVVSVLTVLHQDWLNGKEYKCKVSNKALPAPIEKTISKAKGQPREPQVYTDPPSREKMTKNQVSLKCLVEGFYPSDIAVEWESNGQPENNYKTTPPVLDSDGSFFLYSKLTVDKSRWQQGNVFSCSVMHEALHNHYTQKSLSLSPG

SEQ ID NO: 22 - protein, 329 aa, synthetic construct
ASTKGPSVFPLAPSSKSTSGGTAALGCLVKDYFPEPVTVSWNSGALTSGVHTFPAVLQSSGLYSLSSVVTVPSSSLGTQTYICNVNHKPSNTKVDKRVEPKSCDKTHTCPPCPAPELLGGPSVFLFPPKPKDTLMISRTPEVTCVVVDVSHEDPEVKFNWYVDGVEVHNAKTKPREEQYNSTYRVVSVLTVLHQDWLNGKEYKCKVSNKALPAPIEKTISKAKGQPREPQVYTLPPSRKEMTKNQVSLWCLVKGFYPSDIAVEWESNGQPENNYDTTPPVLKSDGSFFLASDLTVDKSRWQQGNVFSCSVMHEALHNHYTQKSLSLSPG

SEQ ID NO: 23 - protein, 329 aa, synthetic construct
ASTKGPSVFPLAPSSKSTSGGTAALGCLVKDYFPEPVTVSWNSGALTSGVHTFPAVLQSSGLYSLSSVVTVPSSSLGTQTYICNVNHKPSNTKVDKRVEPKSCDKTHTCPPCPAPELLGGPSVFLFPPKPKDTLMISRTPEVTCVVVDVSHEDPEVKFNWYVDGVEVHNAKTKPREEQYNSTYRVVSVLTVLHQDWLNGKEYKCKVSNKALPAPIEKTISKAKGQPREPQVYTLPPSREEMTKNQVSLTCLVKGFYPSDIAVEWESNGQPENNYKTTPPVLDSDGSFFLYSKLTVDKSRWQQGNVFSCSVMHGALHNHYTQKSLSLSPG

SEQ ID NO: 24 - protein, 325 aa, Homo sapiens
ASTKGPSVFPLAPCSRSTSESTAALGCLVKDYFPEPVTVSWNSGALTSGVHTFPAVLQSSGLYSLSSVVTVPSSNFGTQTYTCNVDHKPSNTKVDKTVERKCCVECPPCPAPPVAGPSVFLFPPKPKDTLMISRTPEVTCVVVDVSHEDPEVQFNWYVDGVEVHNAKTKPREEQFNSTFRVVSVLTVVHQDWLNGKEYKCKVSNKGLPAPIEKTISKTKGQPREPQVYTLPPSREEMTKNQVSLTCLVKGFYPSDIAVEWESNGQPENNYKTTPPMLDSDGSFFLYSKLTVDKSRWQQGNVFSCSVMHEALHNHYTQKSLSLSPG

SEQ ID NO: 25 - protein, 376 aa, Homo sapiens
ASTKGPSVFPLAPCSRSTSGGTAALGCLVKDYFPEPVTVSWNSGALTSGVHTFPAVLQSSGLYSLSSVVTVPSSSLGTQTYTCNVNHKPSNTKVDKRVELKTPLGDTTHTCPRCPEPKSCDTPPPCPRCPEPKSCDTPPPCPRCPEPKSCDTPPPCPRCPAPELLGGPSVFLFPPKPKDTLMISRTPEVTCVVVDVSHEDPEVQFKWYVDGVEVHNAKTKPREEQYNSTFRVVSVLTVLHQDWLNGKEYKCKVSNKALPAPIEKTISKTKGQPREPQVYTLPPSREEMTKNQVSLTCLVKGFYPSDIAVEWESSGQPENNYNTTPPMLDSDGSFFLYSKLTVDKSRWQQGNIFSCSVMHEALHNRFTQKSLSLSPG

SEQ ID NO: 26 - protein, 326 aa, Homo sapiens
ASTKGPSVFPLAPCSRSTSESTAALGCLVKDYFPEPVTVSWNSGALTSGVHTFPAVLQSSGLYSLSSVVTVPSSSLGTKTYTCNVDHKPSNTKVDKRVESKYGPPCPSCPAPEFLGGPSVFLFPPKPKDTLMISRTPEVTCVVVDVSQEDPEVQFNWYVDGVEVHNAKTKPREEQFNSTYRVVSVLTVLHQDWLNGKEYKCKVSNKGLPSSIEKTISKAKGQPREPQVYTLPPSQEEMTKNQVSLTCLVKGFYPSDIAVEWESNGQPENNYKTTPPVLDSDGSFFLYSRLTVDKSRWQEGNVFSCSVMHEALHNHYTQKSLSLSLG

SEQ ID NO: 27 - protein, 329 aa, synthetic construct; identical to SEQ ID NO: 23

SEQ ID NO: 28 - protein, 329 aa, synthetic construct
ASTKGPSVFPLAPSSKSTSGGTAALGCLVKDYFPEPVTVSWNSGALTSGVHTFPAVLQSSGLYSLSSVVTVPSSSLGTQTYICNVNHKPSNTKVDKRVEPKSCDKTHTCPPCPAPELLGGPSVFLFPPKPKDTLMISRTPEVTCVVVDVSHEDPEVKFNWYVDGVEVHNAKTKPREEQYNSTYRVVSVLTVLHQDWLNGKEYKCKVSNKALPAPIEKTISKAKGQPRKPQVYTLPPSREEMTKNQVSLTCLVKGFYPSDIAVEWESNGQPENNYKTTPPVLDSDGSFFLYSKLTVDKSRWQQGNVFSCSVMHEALHNHYTQKSLSLSPG

SEQ ID NO: 29 - protein, 329 aa, synthetic construct
ASTKGPSVFPLAPSSKSTSGGTAALGCLVKDYFPEPVTVSWNSGALTSGVHTFPAVLQSSGLYSLSSVVTVPSSSLGTQTYICNVNHKPSNTKVDKRVEPKSCDKTHTCPPCPAPELLGGPSVFLFPPKPKDTLMISRTPEVTCVVVDVSHEDPEVKFNWYVDGVEVHNAKTKPREEQYNSTYRVVSVLTVLHQDWLNGKEYKCKVSNKALPAPIEKTISKAKGQPRRPQVYTLPPSREEMTKNQVSLTCLVKGFYPSDIAVEWESNGQPENNYKTTPPVLDSDGSFFLYSKLTVDKSRWQQGNVFSCSVMHEALHNHYTQKSLSLSPG

SEQ ID NO: 30 - protein, 329 aa, synthetic construct
ASTKGPSVFPLAPSSKSTSGGTAALGCLVKDYFPEPVTVSWNSGALTSGVHTFPAVLQSSGLYSLSSVVTVPSSSLGTQTYICNVNHKPSNTKVDKRVEPKSCDKTHTCPPCPAPELLGGPSVFLFPPKPKDTLMISRTPEVTCVVVDVSHEDPEVKFNWYVDGVEVHNAKTKPREEQYNSTYRVVSVLTVLHQDWLNGKEYKCKVSNKALPAPIEKTISKAKGQPREPQVYTLPPSRKEMTKNQVSLTCLVKGFYPSDIAVEWESNGQPENNYDTTPPVLKSDGSFFLYSDLTVDKSRWQQGNVFSCSVMHGALHNHYTQKSLSLSPG

SEQ ID NO: 31 - protein, 329 aa, synthetic construct
ASTKGPSVFPLAPSSKSTSGGTAALGCLVKDYFPEPVTVSWNSGALTSGVHTFPAVLQSSGLYSLSSVVTVPSSSLGTQTYICNVNHKPSNTKVDKRVEPKSCDKTHTCPPCPAPELLGGPSVFLFPPKPKDTLMISRTPEVTCVVVDVSHEDPEVKFNWYVDGVEVHNAKTKPREEQYNSTYRVVSVLTVLHQDWLNGKEYKCKVSNKALPAPIEKTISKAKGQPREPRVYTLPPSREEMTENQVSLTCLVKGFYPSDIAVEWESNGQPENNYKTTPPVLVSDGSFTLYSWLTVDKSRWQQGNVFSCSVMHGALHNHYTQKSLSLSPG

SEQ ID NO: 32 - protein, 329 aa, synthetic construct
ASTKGPSVFPLAPSSKSTSGGTAALGCLVKDYFPEPVTVSWNSGALTSGVHTFPAVLQSSGLYSLSSVVTVPSSSLGTQTYICNVNHKPSNTKVDKRVEPKSCDKTHTCPPCPAPELLGGPSVFLFPPKPKDTLMISRTPEVTCVVVDVSHEDPEVKFNWYVDGVEVHNAKTKPREEQYNSTYRVVSVLTVLHQDWLNGKEYKCKVSNKALPAPIEKTISKAKGQPRKPRVYTLPPSREEMTENQVSLTCLVKGFYPSDIAVEWESNGQPENNYKTTPPVLVSDGSFTLYSWLTVDKSRWQQGNVFSCSVMHEALHNHYTQKSLSLSPG

SEQ ID NO: 33 - protein, 329 aa, synthetic construct
ASTKGPSVFPLAPSSKSTSGGTAALGCLVKDYFPEPVTVSWNSGALTSGVHTFPAVLQSSGLYSLSSVVTVPSSSLGTQTYICNVNHKPSNTKVDKRVEPKSCDKTHTCPPCPAPELLGGPSVFLFPPKPKDTLMISRTPEVTCVVVDVSHEDPEVKFNWYVDGVEVHNAKTKPREEQYNSTYRVVSVLTVLHQDWLNGKEYKCKVSNKALPAPIEKTISKAKGQPRKPQVYTLPPSRKEMTKNQVSLTCLVKGFYPSDIAVEWESNGQPENNYDTTPPVLKSDGSFFLYSDLTVDKSRWQQGNVFSCSVMHEALHNHYTQKSLSLSPG

SEQ ID NO: 34 - protein, 329 aa, synthetic construct
ASTKGPSVFPLAPSSKSTSGGTAALGCLVKDYFPEPVTVSWNSGALTSGVHTFPAVLQSSGLYSLSSVVTVPSSSLGTQTYICNVNHKPSNTKVDKRVEPKSCDKTHTCPPCPAPELLGGPSVFLFPPKPKDTLMISRTPEVTCVVVDVSHEDPEVKFNWYVDGVEVHNAKTKPREEQYNSTYRVVSVLTVLHQDWLNGKEYKCKVSNKALPAPIEKTISKAKGQPRRPQVYTLPPSREQMTKNQVKLTCDVSGFYPSDIAVEWESNGQPENNYKTTPPVLDSDGSFFLYSKLTVDKSRWQQGNVFSCSVMHEALHNHYTQKSLSLSPG

SEQ ID NO: 35 - protein, 329 aa, synthetic construct
ASTKGPSVFPLAPSSKSTSGGTAALGCLVKDYFPEPVTVSWNSGALTSGVHTFPAVLQSSGLYSLSSVVTVPSSSLGTQTYICNVNHKPSNTKVDKRVEPKSCDKTHTCPPCPAPELLRGPSVFLFPPKPKDTLMISRTPEVTCVVVDVSHEDPEVKFNWYVDGVEVHNAKTKPREEQYNSTYRVVSVLTVLHQDWLNGKEYKCKVSNKALPAPIEKTISKAKGQPRRPQVYTLPPSREEMTKNQVSLTCLVKGFYPSDIAVEWESNGQPENNYKTTPPVLDSDGSFFLYSKLTVDKSRWQQGNVFSCSVMHEALHNHYTQESLSLSPG

SEQ ID NO: 36 - protein, 329 aa, synthetic construct
ASTKGPSVFPLAPSSKSTSGGTAALGCLVKDYFPEPVTVSWNSGALTSGVHTFPAVLQSSGLYSLSSVVTVPSSSLGTQTYICNVNHKPSNTKVDKRVEPKSCDKTHTCPPCPAPELLGAPSVFLFPPKPKDTLMISRTPEVTCVVVDVSHEDPEVKFNWYVDGVEVHNAKTKPREEQYNSTYRVVSVLTVLHQDWLNGKEYKCKVSNKALPAPIEKTISKAKGQPRRPQVYTLPPSREEMTKNQVSLTCLVKGFYPSDIAVEWESNGQPENNYKTTPPVLDSDGSFFLYSKLTVDKSRWQQGNVFSCSVMHEALHNHYTQKKLSLSPG